European Patent Application EP 4 506 457 A1, published February 12, 2025. Title: Anti-CD39 antibody. Applicant: BrightPath Biotherapeutics Co., Ltd. The sequence listing filed with the application follows.

SEQUENCE LISTING (100 sequences)

SEQ ID NO: 1 - protein, 8 aa, Mus musculus
GFSIKDTY

SEQ ID NO: 2 - protein, 8 aa, Mus musculus
IDPANVNT

SEQ ID NO: 3 - protein, 14 aa, Mus musculus
ALYGYDDDAYYFDY

SEQ ID NO: 4 - protein, 10 aa, Mus musculus
ESVDNYGISF

SEQ ID NO: 5 - skipped

SEQ ID NO: 6 - protein, 9 aa, Mus musculus
QQSKEVPYT

SEQ ID NO: 7 - protein, 8 aa, Mus musculus
GYSFTDYN

SEQ ID NO: 8 - protein, 8 aa, Mus musculus
IDPYSGGT

SEQ ID NO: 9 - protein, 14 aa, Mus musculus
GLYGYDDDANYFDD

SEQ ID NO: 10 - protein, 5 aa, Mus musculus
SSVSY

SEQ ID NO: 11 - skipped

SEQ ID NO: 12 - protein, 9 aa, Mus musculus
QQRSSYPLT

SEQ ID NO: 13 - protein, 5 aa, Mus musculus
NYGVH

SEQ ID NO: 14 - protein, 16 aa, Mus musculus
VILRRGSTDYNAAFMS

SEQ ID NO: 15 - protein, 11 aa, Mus musculus
TAVVAGDYFDY

SEQ ID NO: 16 - protein, 11 aa, Mus musculus
KASQNVGTNVA

SEQ ID NO: 17 - protein, 7 aa, Mus musculus
SASYRYS

SEQ ID NO: 18 - protein, 9 aa, Mus musculus
QQYNSYPLT

SEQ ID NO: 19 - protein, 5 aa, Mus musculus
NYGMN

SEQ ID NO: 20 - protein, 17 aa, Mus musculus
WINTYTGEPTYADDFKG

SEQ ID NO: 21 - protein, 14 aa, Mus musculus
KGYYGYPNYYAMDY

SEQ ID NO: 22 - protein, 11 aa, Mus musculus
KASQNVGTAVA

SEQ ID NO: 23 - protein, 7 aa, Mus musculus
SASNRYT

SEQ ID NO: 24 - protein, 9 aa, Mus musculus
QQYSSYPIT

SEQ ID NO: 25 - protein, 5 aa, Mus musculus
SYGVH

SEQ ID NO: 26 - protein, 16 aa, Mus musculus
VIWRRGSTDYNAAFMS

SEQ ID NO: 27 - protein, 11 aa, Mus musculus
GISTATSWFAY

SEQ ID NO: 28 - protein, 11 aa, Mus musculus
KASQNVGTNVA

SEQ ID NO: 29 - protein, 7 aa, Mus musculus
SASYRYS

SEQ ID NO: 30 - protein, 9 aa, Mus musculus
QQYNSYPLT

SEQ ID NO: 31 - protein, 5 aa, Mus musculus
SYGVH

SEQ ID NO: 32 - protein, 16 aa, Mus musculus
VIWRRGSTDYNAAFMS

SEQ ID NO: 33 - protein, 8 aa, Mus musculus
VRGDAMDY

SEQ ID NO: 34 - protein, 11 aa, Mus musculus
KASQNVGTNVA

SEQ ID NO: 35 - protein, 7 aa, Mus musculus
SASYRYS

SEQ ID NO: 36 - protein, 9 aa, Mus musculus
QQYNSYPLT

SEQ ID NO: 37 - protein, 5 aa, Mus musculus
DYGMH

SEQ ID NO: 38 - protein, 17 aa, Mus musculus
YISSGSSIIYYADTVKG

SEQ ID NO: 39 - protein, 9 aa, Mus musculus
KDYPYAMDY

SEQ ID NO: 40 - protein, 11 aa, Mus musculus
KASQNVGTNVA

SEQ ID NO: 41 - protein, 7 aa, Mus musculus
WASNRFT

SEQ ID NO: 42 - protein, 9 aa, Mus musculus
QQYSSSPYT

SEQ ID NO: 43 - protein, 121 aa, Mus musculus
QVQLKQSGAELVKPGASVKLSCTASGFSIKDTYVHWVKQRPEQGLEWIGKIDPANVNTKFDPKFQGKATITADTSSNTAYLQLSSLTSEDTAVYYCALYGYDDDAYYFDYWGQGTTLTVSS

SEQ ID NO: 44 - protein, 111 aa, Mus musculus
NIVLTQSPASLAVSLGQRATISCRASESVDNYGISFMNWFQQKPGQPPKLLIYAASNQGSGVPARFSGSGSGTDFSLNIHPLEEDDTAMYFCQQSKEVPYTFGGGTKLELK

SEQ ID NO: 45 - protein, 121 aa, Mus musculus
EVQLQQSGPELEKPGASVKISCKVSGYSFTDYNLNWVKQYNGKNLEWIGNIDPYSGGTRYNQKFKGKATLTIDQSSSTAYMHLKSLTSEDSAVYYCGLYGYDDDANYFDDWGQGTTLTVSS

SEQ ID NO: 46 - protein, 106 aa, Mus musculus
EIVLTQSPAIMSPSPGEKVTIACSASSSVSYMHWFQQKPGTSPKLWIYATSNLASGVPARFSGSGSGTSYSLTISRMEAEDVATYYCQQRSSYPLTFGAGTKLELK

SEQ ID NO: 47 - protein, 119 aa, Mus musculus
QVQLKESGPSLVQPSQSLSITCTVSGFSLTNYGVHWVRQSPGKGLEWLGVILRRGSTDYNAAFMSRLSITKDNSKSQVFFKMNSLQADDTAIYYCAKTAVVAGDYFDYWGQGTTLTVSS

SEQ ID NO: 48 - protein, 107 aa, Mus musculus
DIVMTQSHKFMSTSVGDRVSVTCKASQNVGTNVAWYQQKPGQSPKALIYSASYRYSGVPDRFTGSGSGTDFTLTISNVQSEDLAEYFCQQYNSYPLTFGTGTKLEIK

SEQ ID NO: 49 - protein, 123 aa, Mus musculus
QIQLVQSGPELKKPGETVKISCEASGYTFINYGMNWVKQAPGKGLKWMGWINTYTGEPTYADDFKGRFAFSLETSANTAYLQINNLKNEDTATYFCARKGYYGYPNYYAMDYWGQGTSVTVSS

SEQ ID NO: 50 - protein, 107 aa, Mus musculus
DIVMTQSQKFMSTSVGDRVSITCKASQNVGTAVAWYQQKPGQSPKLLIYSASNRYTGVPDRFTGSGSGTDFTLTISNMQSEDLADYFCQQYSSYPITFGTGTKLEIK

SEQ ID NO: 51 - protein, 119 aa, Mus musculus
DVQLQESGPSLVQPSQSLSINCTVSGFSLSSYGVHWVRQSPGKGLEWLGVIWRRGSTDYNAAFMSRLSITKDNSKSQVFFKMNRLQADDTATYYCAKGISTATSWFAYWGQGTLVTVSA

SEQ ID NO: 52 - protein, 107 aa, Mus musculus
DIVMTQSHKFMSTSVGDRVSVTCKASQNVGTNVAWYQQKPGQSPKALIYSASYRYSGVPDRFTGSGSGTDFTLTISNVQSEDLAEYFCQQYNSYPLTFGAGTKLELK

SEQ ID NO: 53 - protein, 116 aa, Mus musculus
QVQLKQSGPGLVQPSQSLSITCTVSGFSLTSYGVHWVRQSPGKGLEWLGVIWRRGSTDYNAAFMSRLSITKDTSKSQVFFKMNSLQTDDTAIYYCAGVRGDAMDYWGQGTSVTVSS

SEQ ID NO: 54 - protein, 107 aa, Mus musculus
DIVMTQSHKSMSTSVGDRVSVTCKASQNVGTNVAWYQQKPGQSPKALIYSASYRYSGVPDRFTGSGSGTDFTLTISNVQSEDLAEYFCQQYNSYPLTFGGGTKLEIK

SEQ ID NO: 55 - protein, 118 aa, Mus musculus
EVQLVESGGGLVKPGGSRKLSCAASGFTFSDYGMHWVRQAPEKGLEWVAYISSGSSIIYYADTVKGRFTISRDNAKNTLFLQMTGLRSEDTAMYYCARKDYPYAMDYWGQGTSLAVSS

SEQ ID NO: 56 - protein, 107 aa, Mus musculus; identical to SEQ ID NO: 54

SEQ ID NO: 57 - protein, 121 aa, synthetic construct
  REGION 1..121: note = Humanized sequence
QVQLLQSGAEVKKPGATVKISCKVSGFSIKDTYVHWVRQPPEQGLEWIGKIDPANVNTKFDPKFQGRLTITADTSKNTAYLELSSLRSEDTAVYYCALYGYDDDAYYFDYWGQGTLLTVSS

SEQ ID NO: 58 - protein, 111 aa, synthetic construct
  REGION 1..111: note = Humanized sequence
DIVLTQSPATLALSVGQRATLSCRASESVDNYGISFMNWFQQKPGQPPRLLIYAASNQGSGIPARFSGSGSGTDFTLTINPLESEDFAVYYCQQSKEVPYTFGPGTKLEIK

SEQ ID NO: 59 - protein, 121 aa, synthetic construct
  REGION 1..121: note = Humanized sequence
QVQLVQSGAELVKPGASVKLSCKASGFSIKDTYVHWVKQAPGKGLEWIGKIDPANVNTKFDPKFQGRVTITADTSTNTAYLQLSSLRSEDTAVYYCALYGYDDDAYYFDYWGQGTLVTVSS

SEQ ID NO: 60 - protein, 111 aa, synthetic construct
  REGION 1..111: note = Humanized sequence
EIVLTQSPASLSVSPGERATISCRASESVDNYGISFMNWFQQKPGQAPKLLIYAASNQGSGVPARFSGSGSGTDFTLTISSLEPEDFAVYYCQQSKEVPYTFGQGTKLEIK

SEQ ID NO: 61 - protein, 121 aa, synthetic construct
  REGION 1..121: note = Humanized sequence
QVQLVQSGAELVKPGASVKLSCAASGFSIKDTYVHWVRQAPGKGLEWVGKIDPANVNTKFDPKFQGRFTITADTSKNTAYLQLSSLRSEDTAVYYCALYGYDDDAYYFDYWGQGTLVTVSS

SEQ ID NO: 62 - protein, 111 aa, synthetic construct
  REGION 1..111: note = Humanized sequence
DIVLTQSPASLSVSPGDRATISCRASESVDNYGISFMNWFQQKPGQAPKLLIYAASNQGSGVPARFSGSGSGTDFTLTISSLEPEDFAVYYCQQSKEVPYTFGQGTKLEIK

SEQ ID NO: 63 - protein, 121 aa, synthetic construct
  REGION 1..121: note = Humanized sequence
QVQLLQSGAEVVKPGATVKISCKVSGFSIKDTYVHWVRQPPGQGLEWIGKIDPANVNTKFDPKFQGRFTITADTSINTAYLELSSLTSEDTAVYYCALYGYDDDAYYFDYWGQGTLVTVSS

SEQ ID NO: 64 - protein, 111 aa, synthetic construct
  REGION 1..111: note = Humanized sequence
NIVLTQSPATLSLSLGQRATISCRASESVDNYGISFMNWFQQKPGQPPQLLIYAASNQGSGIPARFSGSGSGTDFTLNINPLESEDFAVYYCQQSKEVPYTFGPGTKLEIK

SEQ ID NO: 65 - protein, 121 aa, synthetic construct
  REGION 1..121: note = Humanized sequence
QVQLQQSGAELKKPGASVKISCKVSGFSIKDTYVHWVRQPPGKGLEWIGKIDPANVNTKFDPKFQGRFTITADTSTDTAYLELSSLRSEDTAVYYCALYGYDDDAYYFDYWGQGTMLTVSS

SEQ ID NO: 66 - protein, 111 aa, synthetic construct
  REGION 1..111: note = Humanized sequence
DIVLTQSPATLSLSLGQRATLSCRASESVDNYGISFMNWFQQKPGQPPRLLIYAASNQGSGIPARFSGSGSGTDFTLNITPLESEDFAVYYCQQSKEVPYTFGPGTKLELK

SEQ ID NO: 67 - protein, 121 aa, synthetic construct
  REGION 1..121: note = Humanized sequence
QVQLLQSGAEVVKPGATVKISCKVSGFSIKDTYVHWVRQRPERGLEWIGKIDPANVNTKFDPKFQGRLTITADTSTDTAYLELSSLRSEDTAVYYCALYGYDDDAYYFDYWGQGTLLTVSS

SEQ ID NO: 68 - protein, 111 aa, synthetic construct
  REGION 1..111: note = Humanized sequence
DIVLTQSPATLSLSPGQRATISCRASESVDNYGISFMNWFQQKPGQPPRLLIYAASNQGSGIPARFSGSGSGTDFTLNIHPLESEDFAVYYCQQSKEVPYTFGPGTKLEIK

SEQ ID NO: 69 - protein, 121 aa, synthetic construct
  REGION 1..121: note = Humanized sequence
EVQLLQSGPEVVKPGATVKISCKVSGYSFTDYNLNWVKQPPGKNLEWIGNIDPYSGGTRYNQKFKGRFTITIDQSINTAYMELRSLTSEDTAVYYCGLYGYDDDANYFDDWGQGTMLTVSS

SEQ ID NO: 70 - protein, 106 aa, synthetic construct
  REGION 1..106: note = Humanized sequence
EIVLTQSPAILSPSPGERVTLNCSASSSVSYMHWFQQKPGQAPRLWIYATSNLASGIPARFSGSGSGTEYTLTISRMESEDFAVYYCQQRSSYPLTFGQGTKLEIK

SEQ ID NO: 71 - protein, 121 aa, synthetic construct
  REGION 1..121: note = Humanized sequence
EVQLVQSGAELKKPGASVKISCKVSGYSFTDYNLNWVKQAPGKGLEWIGNIDPYSGGTRYNQKFKGRVTITIDQSTSTAYMELSSLRSEDTAVYYCGLYGYDDDANYFDDWGQGTLVTVSS

SEQ ID NO: 72 - protein, 106 aa, synthetic construct
  REGION 1..106: note = Humanized sequence
EIVLTQSPATLSLSPGERATISCSASSSVSYMHWFQQKPGQAPKLWIYATSNLASGVPARFSGSGSGTDYTLTISSMEPEDFAVYYCQQRSSYPLTFGGGTKVEIK

SEQ ID NO: 73 - protein, 121 aa, synthetic construct
  REGION 1..121: note = Humanized sequence
EVQLVQSGGELVKPGASVKISCKVSGYSFTDYNLNWVRQAPGKGLEWVGNIDPYSGGTRYNQKFKGRFTITIDQSKNTAYMQLNSLRSEDTAVYYCGLYGYDDDANYFDDWGQGTLVTVSS

SEQ ID NO: 74 - protein, 106 aa, synthetic construct
  REGION 1..106: note = Humanized sequence
EIVLTQSPASLSASPGERVTISCSASSSVSYMHWFQQKPGQAPKLWIYATSNLASGVPARFSGSGSGTDYTLTISSMEPEDFATYYCQQRSSYPLTFGQGTKVEIK

SEQ ID NO: 75 - protein, 121 aa, synthetic construct
  REGION 1..121: note = Humanized sequence
EVQLVQSGPEVKKPGATVKISCKVSGYSFTDYNLNWVKQPPGKNLEWIGNIDPYSGGTRYNQKFKGRFTITIDQSINTAYMHLRSLRSEDTAVYYCGLYGYDDDANYFDDWGQGTMLTVSS

SEQ ID NO: 76 - protein, 106 aa, synthetic construct
  REGION 1..106: note = Humanized sequence
EIVLTQSPATLSPSPGERVTINCSASSSVSYMHWFQQKPGTPPRLWIYATSNLASGIPARFSGSGSGTEYTLTISSMESEDFAVYYCQQRSSYPLTFGPGTKVEIK

SEQ ID NO: 77 - protein, 121 aa, synthetic construct
  REGION 1..121: note = Humanized sequence
EVQLLQSGPEVVKPGATVKISCKVSGYSFTDYNLNWVRQYPGKNLEWVGNIDPYSGGTRYNQKFKGRFTITIDQSKNTAYMELRSLTSEDTAVYYCGLYGYDDDANYFDDWGQGTMLTVSS

SEQ ID NO: 78 - protein, 106 aa, synthetic construct
  REGION 1..106: note = Humanized sequence
EIVLTQSPAILSLSPGERVTITCSASSSVSYMHWFQQKPGQAPRLWIYATSNLASGIPARFSGSGSGTEYTLTISSMESEDFAVYYCQQRSSYPLTFGQGTKLEIK

SEQ ID NO: 79 - protein, 121 aa, synthetic construct
  REGION 1..121: note = Humanized sequence
EVQLLQSGAEVVKPGATVKISCKVSGYSFTDYNLNWVKQPNGKNLEWIGNIDPYSGGTRYNQKFKGRFTITIDQSINTAYMQLNSLRSEDTAVYYCGLYGYDDDANYFDDWGQGTLLTVSS

SEQ ID NO: 80 - protein, 106 aa, synthetic construct
  REGION 1..106: note = Humanized sequence
EIVLTQSPAILSPSPGERVTLTCSASSSVSYMHWFQQKPGKPPRLWIYATSNLASGIPARFSGSGSGTEYTLTISRMESEDFAVYYCQQRSSYPLTFGQGTKLEIK

SEQ ID NO: 81 - protein, 119 aa, synthetic construct
  REGION 1..119: note = Humanized sequence
EVQLVESGGALVQPGRSLRLSCAVSGFTLSNYGVHWVRQAPGKGLEWVAVILRRGSTDYNAAFMSRFTISKDNSKNTVYLQMNSLRADDTAVYYCAKTAVVAGDYFDYWGQGTTVTVSS

SEQ ID NO: 82 - protein, 107 aa, synthetic construct
  REGION 1..107: note = Humanized sequence
DIVMTQSQKFMSTSVGDRVSITCKASQNVGTNVAWYQQKPGQSPKLLIYSASYRYSGVPDRFTGSGSGTDFTLTISNMQSEDLADYFCQQYNSYPLTFGGGTKLEIK

SEQ ID NO: 83 - protein, 119 aa, synthetic construct
  REGION 1..119: note = Humanized sequence
QVQLVESGGGVVQPGGSLRLSCVVSGFTLTNYGVHWVRQAPGKGLEWLAVILRRGSTDYNAAFMSRLAISKDNSKNTVYLELNSLRLDDTAVYYCAKTAVVAGDYFDYWGQGTTVTVSS

SEQ ID NO: 84 - protein, 107 aa, synthetic construct; identical to SEQ ID NO: 82
  REGION 1..107: note = Humanized sequence

SEQ ID NO: 85 - protein, 119 aa, synthetic construct
  REGION 1..119: note = Humanized sequence
QVQLVESGGGVVQPGGSLRLSCVVSGFSLTNYGVHWVRQAPGKGLEWLGVILRRGSTDYNAAFMSRLAISKDNSKNTVYLELNSLRLDDTAVYYCAKTAVVAGDYFDYWGQGTTVTVSS

SEQ ID NO: 86 - protein, 107 aa, synthetic construct; identical to SEQ ID NO: 82
  REGION 1..107: note = Humanized sequence

SEQ ID NO: 87 - protein, 107 aa, Homo sapiens [sequence omitted]

SEQ ID NO: 88 - protein, 330 aa, Homo sapiens
ASTKGPSVFPLAPSSKSTSGGTAALGCLVKDYFPEPVTVSWNSGALTSGVHTFPAVLQSSGLYSLSSVVTVPSSSLGTQTYICNVNHKPSNTKVDKKVEPKSCDKTHTCPPCPAPELLGGPSVFLFPPKPKDTLMISRTPEVTCVVVDVSHEDPEVKFNWYVDGVEVHNAKTKPREEQYNSTYRVVSVLTVLHQDWLNGKEYKCKVSNKALPAPIEKTISKAKGQPREPQVYTLPPSREEMTKNQVSLTCLVKGFYPSDIAVEWESNGQPENNYKTTPPVLDSDGSFFLYSKLTVDKSRWQQGNVFSCSVMHEALHNHYTQKSLSLSPGK

SEQ ID NO: 89 - protein, 330 aa, Homo sapiens
ASTKGPSVFPLAPSSKSTSGGTAALGCLVKDYFPEPVTVSWNSGALTSGVHTFPAVLQSSGLYSLSSVVTVPSSSLGTQTYICNVNHKPSNTKVDKKVEPKSCDKTHTCPPCPAPEAAGGPSVFLFPPKPKDTLMISRTPEVTCVVVDVSHEDPEVKFNWYVDGVEVHNAKTKPREEQYNSTYRVVSVLTVLHQDWLNGKEYKCKVSNKALPAPIEKTISKAKGQPREPQVYTLPPSREEMTKNQVSLTCLVKGFYPSDIAVEWESNGQPENNYKTTPPVLDSDGSFFLYSKLTVDKSRWQQGNVFSCSVMHEALHNHYTQKSLSLSPGK

SEQ ID NO: 90 - protein, 327 aa, Homo sapiens
ASTKGPSVFPLAPCSRSTSESTAALGCLVKDYFPEPVTVSWNSGALTSGVHTFPAVLQSSGLYSLSSVVTVPSSSLGTKTYTCNVDHKPSNTKVDKRVESKYGPPCPPCPAPEFLGGPSVFLFPPKPKDTLMISRTPEVTCVVVDVSQEDPEVQFNWYVDGVEVHNAKTKPREEQFNSTYRVVSVLTVLHQDWLNGKEYKCKVSNKGLPSSIEKTISKAKGQPREPQVYTLPPSQEEMTKNQVSLTCLVKGFYPSDIAVEWESNGQPENNYKTTPPVLDSDGSFFLYSRLTVDKSRWQEGNVFSCSVMHEALHNHYTQKSLSLSPGK

SEQ ID NO: 91 - protein, 232 aa, Homo sapiens
EPKSCDKTHTCPPCPAPEAAGGPSVFLFPPKPKDTLMISRTPEVTCVVVDVSHEDPEVKFNWYVDGVEVHNAKTKPREEQYNSTYRVVSVLTVLHQDWLNGKEYKCKVSNKALPAPIEKTISKAKGQPREPQVYTLPPSREEMTKNQVSLTCLVKGFYPSDIAVEWESNGQPENNYKTTPPVLDSDGSFFLYSKLTVDKSRWQQGNVFSCSVMHEALHNHYTQKSLSLSPGK

SEQ ID NO: 92 - protein, 107 aa, Mus musculus
RADAAPTVSIFPPSSEQLTSGGASVVCFLNNFYPKDINVKWKIDGSERQNGVLNSWTDQDSKDSTYSMSSTLTLTKDEYERHNSYTCEATHKTSTSPIVKSFNRNEC

SEQ ID NO: 93 - protein, 324 aa, Mus musculus
AKTTPPSVYPLAPGSAAQTNSMVTLGCLVKGYFPEPVTVTWNSGSLSSGVHTFPAVLQSDLYTLSSSVTVPSSTWPSETVTCNVAHPASSTKVDKKIVPRDCGCKPCICTVPEVSSVFIFPPKPKDVLTITLTPKVTCVVVDISKDDPEVQFSWFVDDVEVHTAQTQPREEQFNSTFRSVSELPIMHQDWLNGKEFKCRVNSAAFPAPIEKTISKTKGRPKAPQVYTIPPPKEQMAKDKVSLTCMITDFFPEDITVEWQWNGQPAENYKNTQPIMDTDGSYFVYSKLNVQKSNWEAGNTFTCSVLHEGLHNHHTEKSLSHSPGK

SEQ ID NO: 94 - protein, 116 aa, Mus musculus
EVQLQQSGPELVKPGASVKMSCKASGYTFTDYNMHWVKQSHGRTLEWIGYIVPLNGGSTFNQKFKGRATLTVNTSSRTAYMELRSLTSEDSAAYYCARGGTRFAYWGQGTLVTVSA

SEQ ID NO: 95 - protein, 111 aa, Mus musculus
DIVLTQSPASLAVSLGQRATISCRASESVDNFGVSFMYWFQQKPGQPPNLLIYGASNQGSGVPARFRGSGSGTDFSLNIHPMEADDTAMYFCQQTKEVPYTFGGGTKLEIK

SEQ ID NO: 96 - protein, 121 aa, synthetic construct
  REGION 1..121: note = T-31414 VH
QVQLVQSGAEVKKPGASVKVSCKASGYTFKSYEMHWVRQAPGQGLEWMGRINPSVGSTWYAQKFQGRVIMIRDTSTSTVYMELSSLRSEDTAVYYCARGKREGGTEYLRNWGQGTLVTVSS

SEQ ID NO: 97 - protein, 107 aa, synthetic construct
  REGION 1..107: note = T-31414 VL
EIVLIQSPGILSLSPGERATLSCRASQSVSSSYLAWYQQKPGQAPRLLIYGASSRATGIPDRFSGSGSGTDFTLTISRLEPEDFAVYYCQQYHSYITFGGGTKVEIK

SEQ ID NO: 98 - protein, 510 aa, Homo sapiens
MEDTKESNVKTFCSKNILAILGFSSIIAVIALLAVGLTQNKALPENVKYGIVLDAGSSHTSLYIYKWPAEKENDTGVVHQVEECRVKGPGISKFVQKVNEIGIYLTDCMERAREVIPRSQHQETPVYLGATAGMRLLRMESEELADRVLDVVERSLSNYPFDFQGARIITGQEEGAYGWITINYLLGKFSQKTRWFSIVPYETNNQETFGALDLGGASTQVTFVPQNQTIESPDNALQFRLYGKDYNVYTHSFLCYGKDQALWQKLAKDIQVASNEILRDPCFHPGYKKVVNVSDLYKTPCTKRFEMTLPFQQFEIQGIGNYQQCHQSILELFNTSYCPYSQCAFNGIFLPPLQGDFGAFSAFYFVMKFLNLTSEKVSQEKVTEMMKKFCAQPWEEIKTSYAGVKEKYLSEYCFSGTYILSLLLQGYHFTADSWEHIHFIGKIQGSDAGWTLGYMLNLTNMIPAEQPLSTPLSHSTYVFLMVLFSLVLFTVAIIGLLIFHKPSYFWKDMV

SEQ ID NO: 99 - protein, 119 aa, synthetic construct
  REGION 1..119: note = Humanized sequence
QVQLLESGPELVKPSATLSITCTVSGFSLTNYGVHWIRQAPGKGLEWLGVILRRGSTDYNAAFMSRFTISKDNSKNQVYFKLRSVTAEDTAVYYCAKTAVVAGDYFDYWGQGTMVTVSS

SEQ ID NO: 100 - protein, 107 aa, synthetic construct
  REGION 1..107: note = Humanized sequence
DIQMTQSHSTLSLSVGDRVTITCKASQNVGTNVAWYQQKPGQPPKALIYSASYRYSGVPSRFSGSGSGTDFTLTISSVQAEDVAVYYCQQYNSYPLTFGPGTKLEIK